European Patent Application EP 4 209 586 A1, published July 12, 2023. Title: Extracellular vesicle expressing cytokines and antibodies, Method of preparing the same, and Use of the same. Applicant: Daegu Gyeongbuk Institute of Science and Technology Kyungpook National University. The sequence listing filed with the application follows.

SEQUENCE LISTING (17 sequences)

SEQ ID NO: 1 - protein, 153 aa, Artificial Sequence
  IL-2
MYRMQLLSCIALSLALVTNSAPTSSSTKKTQLQLEHLLLDLQMILNGINNYKNPKLTRMLTFKFYMPKKATELKHLQCLEEELKPLEEVLNLAQSKNFHLRPRDLISNINVIVLELKGSETTFMCEYADETATIVEFLNRWITFCQSIISTLT

SEQ ID NO: 2 - protein, 243 aa, Artificial Sequence
  E-scFv
QVQLKQSGPGLVQPSQSLSITCTVSGFSLTNYGVHWVRQSPGKGLEWLGVIWSGGNTDYNTPFTSRLSINKDNSKSQVFFKMNSLQSNDTAIYYCARALTYYDYEFAYWGQGTLVTVSAKLGGGGSGGGGSGGGGSDILLTQSPVILSVSPGERVSFSCRASQSIGTNIHWYQQRTNGSPRLLIKYASESISGIPSRFSGSGSGTDFTLSINSVESEDIADYYCQQNNNWPTTFGAGTKLELK

SEQ ID NO: 3 - protein, 5 aa, Artificial Sequence
  linker-1
GGGGS

SEQ ID NO: 4 - protein, 5 aa, Artificial Sequence
  linker-2
SGGGG

SEQ ID NO: 5 - protein, 5 aa, Artificial Sequence
  linker-3
SRSSG

SEQ ID NO: 6 - protein, 5 aa, Artificial Sequence
  linker-4
SGSSC

SEQ ID NO: 7 - protein, 12 aa, Artificial Sequence
  linker-5
GKSSGSGSESKS

SEQ ID NO: 8 - protein, 6 aa, Artificial Sequence
  linker-6
RPPPPC

SEQ ID NO: 9 - protein, 7 aa, Artificial Sequence
  linker-7
SSPPPPC

SEQ ID NO: 10 - protein, 14 aa, Artificial Sequence
  linker-8
GSTSGSGKSSEGKG

SEQ ID NO: 11 - protein, 18 aa, Artificial Sequence
  linker-9
GSTSGSGKSSEGSGSTKG

SEQ ID NO: 12 - protein, 18 aa, Artificial Sequence
  linker-10
GSTSGSGKPGSGEGSTKG

SEQ ID NO: 13 - protein, 14 aa, Artificial Sequence
  linker-11
EGKSSGSGSESKEF

SEQ ID NO: 14 - DNA, 20 bp, Artificial Sequence
  IL-2-f
agacccagggacttaatcag

SEQ ID NO: 15 - DNA, 20 bp, Artificial Sequence
  IL-2-r
acaatggttgctgtctcatc

SEQ ID NO: 16 - DNA, 15 bp, Artificial Sequence
  Erbituxc-f
ggcccagccggccat

SEQ ID NO: 17 - DNA, 40 bp, Artificial Sequence
  Erbituxc-r
atttaggcccccgaggcctttcagctccagcttggtccca